European Patent Specification EP 3 697 441 B1, published June 7, 2023. Title: Method for generating multispecific antibodies from monospecific antibodies. Applicant: F. Hoffmann-La Roche AG. The sequence listing filed with the application follows.

SEQUENCE LISTING (91 sequences)

SEQ ID NO: 1 - protein, 225 aa, Homo sapiens
DKTHTCPPCPAPELLGGPSVFLFPPKPKDTLMISRTPEVTCVVVDVSHEDPEVKFNWYVDGVEVHNAKTKPREEQYNSTYRVVSVLTVLHQDWLNGKEYKCKVSNKALPAPIEKTISKAKGQPREPQVYTLPPSRDELTKNQVSLTCLVKGFYPSDIAVEWESNGQPENNYKTTPPVLDSDGSFFLYSKLTVDKSRWQQGNVFSCSVMHEALHNHYTQKSLSLSP

SEQ ID NO: 2 - protein, 324 aa, Homo sapiens
ASTKGPSVFPLAPCSRSTSESTAALGCLVKDYFPEPVTVSWNSGALTSGVHTFPAVLQSSGLYSLSSVVTVPSSNFGTQTYTCNVDHKPSNTKVDKTVERKCCVECPPCPAPPVAGPSVFLFPPKPKDTLMISRTPEVTCVVVDVSHEDPEVQFNWYVDGVEVHNAKTKPREEQFNSTFRVVSVLTVVHQDWLNGKEYKCKVSNKGLPAPIEKTISKTKGQPREPQVYTLPPSREEMTKNQVSLTCLVKGFYPSDISVEWESNGQPENNYKTTPPMLDSDGSFFLYSKLTVDKSRWQQGNVFSCSVMHEALHNHYTQKSLSLSP

SEQ ID NO: 3 - protein, 375 aa, Homo sapiens
ASTKGPSVFPLAPCSRSTSGGTAALGCLVKDYFPEPVTVSWNSGALTSGVHTFPAVLQSSGLYSLSSVVTVPSSSLGTQTYTCNVNHKPSNTKVDKRVELKTPLGDTTHTCPRCPEPKSCDTPPPCPRCPEPKSCDTPPPCPRCPEPKSCDTPPPCPRCPAPELLGGPSVFLFPPKPKDTLMISRTPEVTCVVVDVSHEDPEVQFKWYVDGVEVHNAKTKPREEQYNSTFRVVSVLTVLHQDWLNGKEYKCKVSNKALPAPIEKTISKTKGQPREPQVYTLPPSREEMTKNQVSLTCLVKGFYPSDIAVEWESSGQPENNYNTTPPMLDSDGSFFLYSKLTVDKSRWQQGNIFSCSVMHEALHNRFTQKSLSLSP

SEQ ID NO: 4 - protein, 227 aa, Homo sapiens
ESKYGPPCPSCPAPEFLGGPSVFLFPPKPKDTLMISRTPEVTCVVVDVSQEDPEVQFNWYVDGVEVHNAKTKPREEQFNSTYRVVSVLTVLHQDWLNGKEYKCKVSNKGLPSSIEKTISKAKGQPREPQVYTLPPSQEEMTKNQVSLTCLVKGFYPSDIAVEWESNGQPENNYKTTPPVLDSDGSFFLYSRLTVDKSRWQEGNVFSCSVMHEALHNHYTQKSLSLSL

SEQ ID NO: 5 - protein, 225 aa, Artificial Sequence
  human IgG1 Fc-region derived Fc-region polypeptide with the mutations L234A, L235A
DKTHTCPPCPAPEAAGGPSVFLFPPKPKDTLMISRTPEVTCVVVDVSHEDPEVKFNWYVDGVEVHNAKTKPREEQYNSTYRVVSVLTVLHQDWLNGKEYKCKVSNKALPAPIEKTISKAKGQPREPQVYTLPPSRDELTKNQVSLTCLVKGFYPSDIAVEWESNGQPENNYKTTPPVLDSDGSFFLYSKLTVDKSRWQQGNVFSCSVMHEALHNHYTQKSLSLSP

SEQ ID NO: 6 - protein, 225 aa, Artificial Sequence
  human IgG1 Fc-region derived Fc-region polypeptide with Y349C, T366S, L368A and Y407V mutations
DKTHTCPPCPAPELLGGPSVFLFPPKPKDTLMISRTPEVTCVVVDVSHEDPEVKFNWYVDGVEVHNAKTKPREEQYNSTYRVVSVLTVLHQDWLNGKEYKCKVSNKALPAPIEKTISKAKGQPREPQVCTLPPSRDELTKNQVSLSCAVKGFYPSDIAVEWESNGQPENNYKTTPPVLDSDGSFFLVSKLTVDKSRWQQGNVFSCSVMHEALHNHYTQKSLSLSP

SEQ ID NO: 7 - protein, 225 aa, Artificial Sequence
  human IgG1 Fc-region derived Fc-region polypeptide with S354C, T366W mutations
DKTHTCPPCPAPELLGGPSVFLFPPKPKDTLMISRTPEVTCVVVDVSHEDPEVKFNWYVDGVEVHNAKTKPREEQYNSTYRVVSVLTVLHQDWLNGKEYKCKVSNKALPAPIEKTISKAKGQPREPQVYTLPPCRDELTKNQVSLWCLVKGFYPSDIAVEWESNGQPENNYKTTPPVLDSDGSFFLYSKLTVDKSRWQQGNVFSCSVMHEALHNHYTQKSLSLSP

SEQ ID NO: 8 - protein, 225 aa, Artificial Sequence
  human IgG1 Fc-region derived Fc-region polypeptide with L234A, L235A mutations and Y349C, T366S, L368A, Y407V mutations
DKTHTCPPCPAPEAAGGPSVFLFPPKPKDTLMISRTPEVTCVVVDVSHEDPEVKFNWYVDGVEVHNAKTKPREEQYNSTYRVVSVLTVLHQDWLNGKEYKCKVSNKALPAPIEKTISKAKGQPREPQVCTLPPSRDELTKNQVSLSCAVKGFYPSDIAVEWESNGQPENNYKTTPPVLDSDGSFFLVSKLTVDKSRWQQGNVFSCSVMHEALHNHYTQKSLSLSP

SEQ ID NO: 9 - protein, 225 aa, Artificial Sequence
  human IgG1 Fc-region derived Fc-region polypeptide with a L234A, L235A and S354C, T366W mutations
DKTHTCPPCPAPEAAGGPSVFLFPPKPKDTLMISRTPEVTCVVVDVSHEDPEVKFNWYVDGVEVHNAKTKPREEQYNSTYRVVSVLTVLHQDWLNGKEYKCKVSNKALPAPIEKTISKAKGQPREPQVYTLPPCRDELTKNQVSLWCLVKGFYPSDIAVEWESNGQPENNYKTTPPVLDSDGSFFLYSKLTVDKSRWQQGNVFSCSVMHEALHNHYTQKSLSLSP

SEQ ID NO: 10 - protein, 225 aa, Artificial Sequence
  human IgG1 Fc-region derived Fc-region polypeptide with a P329G mutation
DKTHTCPPCPAPELLGGPSVFLFPPKPKDTLMISRTPEVTCVVVDVSHEDPEVKFNWYVDGVEVHNAKTKPREEQYNSTYRVVSVLTVLHQDWLNGKEYKCKVSNKALGAPIEKTISKAKGQPREPQVYTLPPSRDELTKNQVSLTCLVKGFYPSDIAVEWESNGQPENNYKTTPPVLDSDGSFFLYSKLTVDKSRWQQGNVFSCSVMHEALHNHYTQKSLSLSP

SEQ ID NO: 11 - protein, 225 aa, Artificial Sequence
  human IgG1 Fc-region derived Fc-region polypeptide with L234A, L235A mutations and P329G mutation
DKTHTCPPCPAPEAAGGPSVFLFPPKPKDTLMISRTPEVTCVVVDVSHEDPEVKFNWYVDGVEVHNAKTKPREEQYNSTYRVVSVLTVLHQDWLNGKEYKCKVSNKALGAPIEKTISKAKGQPREPQVYTLPPSRDELTKNQVSLTCLVKGFYPSDIAVEWESNGQPENNYKTTPPVLDSDGSFFLYSKLTVDKSRWQQGNVFSCSVMHEALHNHYTQKSLSLSP

SEQ ID NO: 12 - protein, 225 aa, Artificial Sequence
  human IgG1 Fc-region derived Fc-region polypeptide with a P239G mutation and Y349C, T366S, L368A, Y407V mutations
DKTHTCPPCPAPELLGGPSVFLFPPKPKDTLMISRTPEVTCVVVDVSHEDPEVKFNWYVDGVEVHNAKTKPREEQYNSTYRVVSVLTVLHQDWLNGKEYKCKVSNKALGAPIEKTISKAKGQPREPQVCTLPPSRDELTKNQVSLSCAVKGFYPSDIAVEWESNGQPENNYKTTPPVLDSDGSFFLVSKLTVDKSRWQQGNVFSCSVMHEALHNHYTQKSLSLSP

SEQ ID NO: 13 - protein, 225 aa, Artificial Sequence
  human IgG1 Fc-region derived Fc-region polypeptide with a P329G mutation and S354C, T366W mutation
DKTHTCPPCPAPELLGGPSVFLFPPKPKDTLMISRTPEVTCVVVDVSHEDPEVKFNWYVDGVEVHNAKTKPREEQYNSTYRVVSVLTVLHQDWLNGKEYKCKVSNKALGAPIEKTISKAKGQPREPQVYTLPPCRDELTKNQVSLWCLVKGFYPSDIAVEWESNGQPENNYKTTPPVLDSDGSFFLYSKLTVDKSRWQQGNVFSCSVMHEALHNHYTQKSLSLSP

SEQ ID NO: 14 - protein, 225 aa, Artificial Sequence
  human IgG1 Fc-region derived Fc-region polypeptide with L234A, L235A, P329G and Y349C, T366S, L368A, Y407V mutations
DKTHTCPPCPAPEAAGGPSVFLFPPKPKDTLMISRTPEVTCVVVDVSHEDPEVKFNWYVDGVEVHNAKTKPREEQYNSTYRVVSVLTVLHQDWLNGKEYKCKVSNKALGAPIEKTISKAKGQPREPQVCTLPPSRDELTKNQVSLSCAVKGFYPSDIAVEWESNGQPENNYKTTPPVLDSDGSFFLVSKLTVDKSRWQQGNVFSCSVMHEALHNHYTQKSLSLSP

SEQ ID NO: 15 - protein, 225 aa, Artificial Sequence
  human IgG1 Fc-region derived Fc-region polypeptide with L234A, L235A, P329G mutations and S354C, T366W mutations
DKTHTCPPCPAPEAAGGPSVFLFPPKPKDTLMISRTPEVTCVVVDVSHEDPEVKFNWYVDGVEVHNAKTKPREEQYNSTYRVVSVLTVLHQDWLNGKEYKCKVSNKALGAPIEKTISKAKGQPREPQVYTLPPCRDELTKNQVSLWCLVKGFYPSDIAVEWESNGQPENNYKTTPPVLDSDGSFFLYSKLTVDKSRWQQGNVFSCSVMHEALHNHYTQKSLSLSP

SEQ ID NO: 16 - protein, 227 aa, Artificial Sequence
  human IgG4 Fc-region derived Fc-region polypeptide with S228P and L235E mutations
ESKYGPPCPPCPAPEFEGGPSVFLFPPKPKDTLMISRTPEVTCVVVDVSQEDPEVQFNWYVDGVEVHNAKTKPREEQFNSTYRVVSVLTVLHQDWLNGKEYKCKVSNKGLPSSIEKTISKAKGQPREPQVYTLPPSQEEMTKNQVSLTCLVKGFYPSDIAVEWESNGQPENNYKTTPPVLDSDGSFFLYSRLTVDKSRWQEGNVFSCSVMHEALHNHYTQKSLSLSL

SEQ ID NO: 17 - protein, 227 aa, Artificial Sequence
  human IgG4 Fc-region derived Fc-region polypeptide with S228P, L235E mutations and P329G mutation
ESKYGPPCPPCPAPEFEGGPSVFLFPPKPKDTLMISRTPEVTCVVVDVSQEDPEVQFNWYVDGVEVHNAKTKPREEQFNSTYRVVSVLTVLHQDWLNGKEYKCKVSNKGLGSSIEKTISKAKGQPREPQVYTLPPSQEEMTKNQVSLTCLVKGFYPSDIAVEWESNGQPENNYKTTPPVLDSDGSFFLYSRLTVDKSRWQEGNVFSCSVMHEALHNHYTQKSLSLSL

SEQ ID NO: 18 - protein, 227 aa, Artificial Sequence
  human IgG4 Fc-region derived Fc-region polypeptide with S354C, T366W mutations
ESKYGPPCPSCPAPEFLGGPSVFLFPPKPKDTLMISRTPEVTCVVVDVSQEDPEVQFNWYVDGVEVHNAKTKPREEQFNSTYRVVSVLTVLHQDWLNGKEYKCKVSNKGLPSSIEKTISKAKGQPREPQVYTLPPCQEEMTKNQVSLWCLVKGFYPSDIAVEWESNGQPENNYKTTPPVLDSDGSFFLYSRLTVDKSRWQEGNVFSCSVMHEALHNHYTQKSLSLSL

SEQ ID NO: 19 - protein, 227 aa, Artificial Sequence
  human IgG4 Fc-region derived Fc-region polypeptide with Y349C, T366S, L368A, Y407V mutations
ESKYGPPCPSCPAPEFLGGPSVFLFPPKPKDTLMISRTPEVTCVVVDVSQEDPEVQFNWYVDGVEVHNAKTKPREEQFNSTYRVVSVLTVLHQDWLNGKEYKCKVSNKGLPSSIEKTISKAKGQPREPQVCTLPPSQEEMTKNQVSLSCAVKGFYPSDIAVEWESNGQPENNYKTTPPVLDSDGSFFLVSRLTVDKSRWQEGNVFSCSVMHEALHNHYTQKSLSLSL

SEQ ID NO: 20 - protein, 227 aa, Artificial Sequence
  human IgG4 Fc-region derived Fc-region polypeptide with a S228P, L235E and S354C, T366W mutations
ESKYGPPCPPCPAPEFEGGPSVFLFPPKPKDTLMISRTPEVTCVVVDVSQEDPEVQFNWYVDGVEVHNAKTKPREEQFNSTYRVVSVLTVLHQDWLNGKEYKCKVSNKGLPSSIEKTISKAKGQPREPQVYTLPPCQEEMTKNQVSLWCLVKGFYPSDIAVEWESNGQPENNYKTTPPVLDSDGSFFLYSRLTVDKSRWQEGNVFSCSVMHEALHNHYTQKSLSLSL

SEQ ID NO: 21 - protein, 227 aa, Artificial Sequence
  human IgG4 Fc-region derived Fc-region polypeptide with a S228P, L235E and Y349C, T366S, L368A, Y407V mutations
ESKYGPPCPPCPAPEFEGGPSVFLFPPKPKDTLMISRTPEVTCVVVDVSQEDPEVQFNWYVDGVEVHNAKTKPREEQFNSTYRVVSVLTVLHQDWLNGKEYKCKVSNKGLPSSIEKTISKAKGQPREPQVCTLPPSQEEMTKNQVSLSCAVKGFYPSDIAVEWESNGQPENNYKTTPPVLDSDGSFFLVSRLTVDKSRWQEGNVFSCSVMHEALHNHYTQKSLSLSL

SEQ ID NO: 22 - protein, 227 aa, Artificial Sequence
  human IgG4 Fc-region derived Fc-region polypeptide with a P329G mutation
ESKYGPPCPSCPAPEFLGGPSVFLFPPKPKDTLMISRTPEVTCVVVDVSQEDPEVQFNWYVDGVEVHNAKTKPREEQFNSTYRVVSVLTVLHQDWLNGKEYKCKVSNKGLGSSIEKTISKAKGQPREPQVYTLPPSQEEMTKNQVSLTCLVKGFYPSDIAVEWESNGQPENNYKTTPPVLDSDGSFFLYSRLTVDKSRWQEGNVFSCSVMHEALHNHYTQKSLSLSL

SEQ ID NO: 23 - protein, 227 aa, Artificial Sequence
  human IgG4 Fc-region derived Fc-region polypeptide with a P239G and Y349C, T366S, L368A, Y407V mutations
ESKYGPPCPSCPAPEFLGGPSVFLFPPKPKDTLMISRTPEVTCVVVDVSQEDPEVQFNWYVDGVEVHNAKTKPREEQFNSTYRVVSVLTVLHQDWLNGKEYKCKVSNKGLGSSIEKTISKAKGQPREPQVCTLPPSQEEMTKNQVSLSCAVKGFYPSDIAVEWESNGQPENNYKTTPPVLDSDGSFFLVSRLTVDKSRWQEGNVFSCSVMHEALHNHYTQKSLSLSL

SEQ ID NO: 24 - protein, 227 aa, Artificial Sequence
  human IgG4 Fc-region derived Fc-region polypeptide with a P329G and S354C, T366W mutations
ESKYGPPCPSCPAPEFLGGPSVFLFPPKPKDTLMISRTPEVTCVVVDVSQEDPEVQFNWYVDGVEVHNAKTKPREEQFNSTYRVVSVLTVLHQDWLNGKEYKCKVSNKGLGSSIEKTISKAKGQPREPQVYTLPPCQEEMTKNQVSLWCLVKGFYPSDIAVEWESNGQPENNYKTTPPVLDSDGSFFLYSRLTVDKSRWQEGNVFSCSVMHEALHNHYTQKSLSLSL

SEQ ID NO: 25 - protein, 227 aa, Artificial Sequence
  human IgG4 Fc-region derived Fc-region polypeptide with a S228P, L235E, P329G and Y349C, T366S, L368A, Y407V mutations
ESKYGPPCPPCPAPEFEGGPSVFLFPPKPKDTLMISRTPEVTCVVVDVSQEDPEVQFNWYVDGVEVHNAKTKPREEQFNSTYRVVSVLTVLHQDWLNGKEYKCKVSNKGLGSSIEKTISKAKGQPREPQVCTLPPSQEEMTKNQVSLSCAVKGFYPSDIAVEWESNGQPENNYKTTPPVLDSDGSFFLVSRLTVDKSRWQEGNVFSCSVMHEALHNHYTQKSLSLSL

SEQ ID NO: 26 - protein, 227 aa, Artificial Sequence
  human IgG4 Fc-region derived Fc-region polypeptide with a S228P, L235E, P329G and S354C, T366W mutations
ESKYGPPCPPCPAPEFEGGPSVFLFPPKPKDTLMISRTPEVTCVVVDVSQEDPEVQFNWYVDGVEVHNAKTKPREEQFNSTYRVVSVLTVLHQDWLNGKEYKCKVSNKGLGSSIEKTISKAKGQPREPQVYTLPPCQEEMTKNQVSLWCLVKGFYPSDIAVEWESNGQPENNYKTTPPVLDSDGSFFLYSRLTVDKSRWQEGNVFSCSVMHEALHNHYTQKSLSLSL

SEQ ID NO: 27 - protein, 103 aa, Homo sapiens
ASTKGPSVFPLAPSSKSTSGGTAALGCLVKDYFPEPVTVSWNSGALTSGVHTFPAVLQSSGLYSLSSVVTVPSSSLGTQTYICNVNHKPSNTKVDKKVEPKSC

SEQ ID NO: 28 - protein, 107 aa, Homo sapiens
APELLGGPSVFLFPPKPKDTLMISRTPEVTCVWDVSHEDPEVKFNWYVDGVEVHNAKTKPREEQESTYRWSVLTVLHQDWLNGKEYKCKVSNKALPAPIEKTISKAK

SEQ ID NO: 29 - protein, 105 aa, Homo sapiens
GQPREPQVYTLPPSRDELTKNQVSLTCLVKGFYPSDIAVEWESNGQPENNYKTTPPVLDSDGSFFLYSKLTVDKSRWQQGNVFSCSVMHEALHNHYTQKSLSLSP

SEQ ID NO: 30 - protein, 10 aa, Homo sapiens
  MISC_FEATURE (8)..(8): X=S or P
DKTHTCPXCP

SEQ ID NO: 31 - protein, 7 aa, Homo sapiens
  MISC_FEATURE (5)..(5): X=S or P
HTCPXCP

SEQ ID NO: 32 - protein, 5 aa, Homo sapiens
  MISC_FEATURE (3)..(3): X=S or P
CPXCP

SEQ ID NO: 33 - protein, 107 aa, Homo sapiens [sequence omitted]

SEQ ID NO: 34 - protein, 105 aa, Homo sapiens
QPKAAPSVTLFPPSSEELQANKATLVCLISDFYPGAVTVAWKADSSPVKAGVETTTPSKQSNNKYAASSYLSLTPEQWKSHRSYSCQVTHEGSTVEKTVAPTECS

SEQ ID NO: 35 - protein, 240 aa, Artificial Sequence
  MHCFcRP-hole-D356K-His8
DKTHTCPPCPAPELLGGPSVFLFPPKPKDTLMISRTPEVTCVVVDVSHEDPEVKFNWYVDGVEVHNAKTKPREEQYNSTYRVVSVLTVLHQDWLNGKEYKCKVSNKALPAPIEKTISKAKGQPREPQVYTLPPSRKELTKNQVSLSCAVKGFYPSDIAVEWESNGQPENNYKTTPPVLDSDGSFFLVSKLTVDKSRWQQGNVFSCSVMHEALHNHYTQKSLSLSPGKGGGGSHHHHHHHH

SEQ ID NO: 36 - protein, 240 aa, Artificial Sequence
  MHCFcRP-hole-E357K-His8
DKTHTCPPCPAPELLGGPSVFLFPPKPKDTLMISRTPEVTCVVVDVSHEDPEVKFNWYVDGVEVHNAKTKPREEQYNSTYRVVSVLTVLHQDWLNGKEYKCKVSNKALPAPIEKTISKAKGQPREPQVYTLPPSRDKLTKNQVSLSCAVKGFYPSDIAVEWESNGQPENNYKTTPPVLDSDGSFFLVSKLTVDKSRWQQGNVFSCSVMHEALHNHYTQKSLSLSPGKGGGGSHHHHHHHH

SEQ ID NO: 37 - protein, 240 aa, Artificial Sequence
  MHCFcRP-knob-K370E-His8
DKTHTCPPCPAPELLGGPSVFLFPPKPKDTLMISRTPEVTCVVVDVSHEDPEVKFNWYVDGVEVHNAKTKPREEQYNSTYRVVSVLTVLHQDWLNGKEYKCKVSNKALPAPIEKTISKAKGQPREPQVYTLPPSRDELTKNQVSLWCLVEGFYPSDIAVEWESNGQPENNYKTTPPVLDSDGSFFLYSKLTVDKSRWQQGNVFSCSVMHEALHNHYTQKSLSLSPGKGGGGSHHHHHHHH

SEQ ID NO: 38 - protein, 240 aa, Artificial Sequence
  MHCFcRP-knob-K439E-His8
DKTHTCPPCPAPELLGGPSVFLFPPKPKDTLMISRTPEVTCVVVDVSHEDPEVKFNWYVDGVEVHNAKTKPREEQYNSTYRVVSVLTVLHQDWLNGKEYKCKVSNKALPAPIEKTISKAKGQPREPQVYTLPPSRDELTKNQVSLWCLVKGFYPSDIAVEWESNGQPENNYKTTPPVLDSDGSFFLYSKLTVDKSRWQQGNVFSCSVMHEALHNHYTQESLSLSPGKGGGGSHHHHHHHH

SEQ ID NO: 39 - protein, 214 aa, Artificial Sequence
  anti-bio antibody full length light chain
DIQMTQSPSSLSASVGDRVTITCRASGNIHNYLSWYQQKPGKVPKLLIYSAKTLADGVPSRFSGSGSGTDFTLTISSLQPEDVATYYCQHFWSSIYTFGQGTKLEIKRTVAAPSVFIFPPSDEQLKSGTASVVCLLNNFYPREAKVQWKVDNALQSGNSQESVTEQDSKDSTYSLSSTLTLSKADYEKHKVYACEVTHQGLSSPVTKSFNRGEC

SEQ ID NO: 40 - protein, 450 aa, Artificial Sequence
  anti-bio antibody full length heavy chain-knob-cys
QVQLVQSGAEVKKPGSSVKVSCKSSGFNNKDTFFQWVRQAPGQGLEWMGRIDPANGFTKYAQKFQGRVTITADTSTSTAYMELSSLRSEDTAVYYCARWDTYGAAWFAYWGQGTLVTVSSASTKGPSVFPLAPSSKSTSGGTAALGCLVKDYFPEPVTVSWNSGALTSGVHTFPAVLQSSGLYSLSSVVTVPSSSLGTQTYICNVNHKPSNTKVDKKVEPKSCDKTHTCPPCPAPELLGGPSVFLFPPKPKDTLMISRTPEVTCVVVDVSHEDPEVKFNWYVDGVEVHNAKTKPREEQYNSTYRVVSVLTVLHQDWLNGKEYKCKVSNKALPAPIEKTISKAKGQPREPQVYTLPPCRDELTKNQVSLWCLVKGFYPSDIAVEWESNGQPENNYKTTPPVLDSDGSFFLYSKLTVDKSRWQQGNVFSCSVMHEALHNHYTQKSLSLSPGK

SEQ ID NO: 41 - protein, 450 aa, Artificial Sequence
  anti-bio antibody full length heavy chain-hole-cys
QVQLVQSGAEVKKPGSSVKVSCKSSGFNNKDTFFQWVRQAPGQGLEWMGRIDPANGFTKYAQKFQGRVTITADTSTSTAYMELSSLRSEDTAVYYCARWDTYGAAWFAYWGQGTLVTVSSASTKGPSVFPLAPSSKSTSGGTAALGCLVKDYFPEPVTVSWNSGALTSGVHTFPAVLQSSGLYSLSSVVTVPSSSLGTQTYICNVNHKPSNTKVDKKVEPKSCDKTHTCPPCPAPELLGGPSVFLFPPKPKDTLMISRTPEVTCVVVDVSHEDPEVKFNWYVDGVEVHNAKTKPREEQYNSTYRVVSVLTVLHQDWLNGKEYKCKVSNKALPAPIEKTISKAKGQPREPQVCTLPPSRDELTKNQVSLSCAVKGFYPSDIAVEWESNGQPENNYKTTPPVLDSDGSFFLVSKLTVDKSRWQQGNVFSCSVMHEALHNHYTQKSLSLSPGK

SEQ ID NO: 42 - protein, 219 aa, Artificial Sequence
  anti-fluos antibody full length light chain
DIVMTQTPLSLSVTPGQPASISCKSSQSLVHSNGNTYLRWYLQKPGQSPKVLIYKVSNRVSGVPDRFSGSGSGTDFTLKISRVEAEDVGVYYCSQSTHVPWTFGQGTKLEIKRTVAAPSVFIFPPSDEQLKSGTASVVCLLNNFYPREAKVQWKVDNALQSGNSQESVTEQDSKDSTYSLSSTLTLSKADYEKHKVYACEVTHQGLSSPVTKSFNRGEC

SEQ ID NO: 43 - protein, 448 aa, Artificial Sequence
  anti-fluos antibody full length heavy chain-knob-cys
GVKLDETGGGLVQPGGAMKLSCVTSGFTFGHYWMNWVRQSPEKGLEWVAQFRNKPYNYETYYSDSVKGRFTISRDDSKSSVYLQMNNLRVEDTGIYYCTGASYGMEYLGQGTSVTVSSASTKGPSVFPLAPSSKSTSGGTAALGCLVKDYFPEPVTVSWNSGALTSGVHTFPAVLQSSGLYSLSSVVTVPSSSLGTQTYICNVNHKPSNTKVDKKVEPKSCDKTHTCPPCPAPELLGGPSVFLFPPKPKDTLMISRTPEVTCVVVDVSHEDPEVKFNWYVDGVEVHNAKTKPREEQYNSTYRVVSVLTVLHQDWLNGKEYKCKVSNKALPAPIEKTISKAKGQPREPQVYTLPPCRDELTKNQVSLWCLVKGFYPSDIAVEWESNGQPENNYKTTPPVLDSDGSFFLYSKLTVDKSRWQQGNVFSCSVMHEALHNHYTQKSLSLSPGK

SEQ ID NO: 44 - protein, 448 aa, Artificial Sequence
  anti-fluos antibody full length heavy chain-hole-cys
GVKLDETGGGLVQPGGAMKLSCVTSGFTFGHYWMNWVRQSPEKGLEWVAQFRNKPYNYETYYSDSVKGRFTISRDDSKSSVYLQMNNLRVEDTGIYYCTGASYGMEYLGQGTSVTVSSASTKGPSVFPLAPSSKSTSGGTAALGCLVKDYFPEPVTVSWNSGALTSGVHTFPAVLQSSGLYSLSSVVTVPSSSLGTQTYICNVNHKPSNTKVDKKVEPKSCDKTHTCPPCPAPELLGGPSVFLFPPKPKDTLMISRTPEVTCVVVDVSHEDPEVKFNWYVDGVEVHNAKTKPREEQYNSTYRVVSVLTVLHQDWLNGKEYKCKVSNKALPAPIEKTISKAKGQPREPQVCTLPPSRDELTKNQVSLSCAVKGFYPSDIAVEWESNGQPENNYKTTPPVLDSDGSFFLVSKLTVDKSRWQQGNVFSCSVMHEALHNHYTQKSLSLSPGK

SEQ ID NO: 45 - protein, 214 aa, Artificial Sequence
  anti-dig antibody full length light chain
DIQMTQSPSSLSASVGDRVTITCRASQDIKNYLNWYQQKPGKAPKLLIYYSSTLLSGVPSRFSGSGSGTDFTLTISSLQPEDFATYYCQQSITLPPTFGGGTKVEIKRTVAAPSVFIFPPSDEQLKSGTASVVCLLNNFYPREAKVQWKVDNALQSGNSQESVTEQDSKDSTYSLSSTLTLSKADYEKHKVYACEVTHQGLSSPVTKSFNRGEC

SEQ ID NO: 46 - protein, 219 aa, Artificial Sequence
  anti-LeY antibody full length light chain
DVLMTQSPLSLPVSLGDQASISCRSSQIIVHSNGNTYLEWYLQKPGQSPKLLIYKVSNRFSGVPDRFSGSGSGTDFTLKISRVEAEDLGVYYCFQGSHVPFTFGSGTKLEIKRTVAAPSVFIFPPSDEQLKSGTASVVCLLNNFYPREAKVQWKVDNALQSGNSQESVTEQDSKDSTYSLSSTLTLSKADYEKHKVYACEVTHQGLSSPVTKSFNRGEC

SEQ ID NO: 47 - protein, 214 aa, Artificial Sequence
  anti-PDGF antibody full length light chain
DIQMTQSPSSLSASVGDRVAITCRASQSISNYLNWYQQKPGKAPKLLIYAASSLQSGVPSRFSGSGSGTDFTLTISSLQPEDFATYYCQQSYSTPLTFGGGTKVEIKRTVAAPSVFIFPPSDEQLKSGTASVVCLLNNFYPREAKVQWKVDNALQSGNSQESVTEQDSKDSTYSLSSTLTLSKADYEKHKVYACEVTHQGLSSPVTKSFNRGEC

SEQ ID NO: 48 - protein, 214 aa, Artificial Sequence
  anti-VEGF antibody full length light chain
DIQLTQSPSSLSASVGDRVTITCSASQDISNYLNWYQQKPGKAPKVLIYFTSSLHSGVPSRFSGSGSGTDFTLTISSLQPEDFATYYCQQYSTVPWTFGQGTKVEIKRTVAAPSVFIFPPSDEQLKSGTASVVCLLNNFYPREAKVQWKVDNALQSGNSQESVTEQDSKDSTYSLSSTLTLSKADYEKHKVYACEVTHQGLSSPVTKSFNRGEC

SEQ ID NO: 49 - protein, 228 aa, Artificial Sequence
  anti-dig antibody VH-CH1 fragment
QVQLVESGGGLVKPGGSLRLSCAASGFTFSDYAMSWIRQAPGKGLEWVSSINIGATYIYYADSVKGRFTISRDNAKNSLYLQMNSLRAEDTAVYYCARPGSPYEYDKAYYSMAYWGQGTTVTVSSASTKGPSVFPLAPSSKSTSGGTAALGCLVKDYFPEPVTVSWNSGALTSGVHTFPAVLQSSGLYSLSSVVTVPSSSLGTQTYICNVNHKPSNTKVDKKVEPKSC

SEQ ID NO: 50 - protein, 222 aa, Artificial Sequence
  anti-LeY antibody VH-CH1 fragment
DVKLVESGGGLVQPGGSLKLSCATSGFTFSDYYMYWVRQTPEKRLEWVAYISNDDSSAAYSDTVKGRFTISRDNARNTLYLQMSRLKSEDTAIYYCARGLAWGAWFAYWGQGTLVTVSSASTKGPSVFPLAPSSKSTSGGTAALGCLVKDYFPEPVTVSWNSGALTSGVHTFPAVLQSSGLYSLSSVVTVPSSSLGTQTYICNVNHKPSNTKVDKKVEPKSC

SEQ ID NO: 51 - protein, 223 aa, Artificial Sequence
  anti-PDGF antibody VH-CH1 fragment
EVQLVESGGGLVQPGGSLRLSCAASGFTFSSYWMSWVRQAPEKGLEWVSTISDGGGLTYYADSVKGRFTISRDNAKNSLYLQMNSLRAEDTAVYYCAESGGYTDWLFGYWGQGTLVTVSSASTKGPSVFPLAPSSKSTSGGTAALGCLVKDYFPEPVTVSWNSGALTSGVHTFPAVLQSSGLYSLSSVVTVPSSSLGTQTYICNVNHKPSNTKVDKKVEPKSC

SEQ ID NO: 52 - protein, 226 aa, Artificial Sequence
  anti-VEGF antibody VH-CH1 fragment
EVQLVESGGGLVQPGGSLRLSCAASGYDFTHYGMNWVRQAPGKGLEWVGWINTYTGEPTYAADFKRRFTFSLDTSKSTAYLQMNSLRAEDTAVYYCAKYPYYYGTSHWYFDVWGQGTLVTVSSASTKGPSVFPLAPSSKSTSGGTAALGCLVKDYFPEPVTVSWNSGALTSGVHTFPAVLQSSGLYSLSSVVTVPSSSLGTQTYICNVNHKPSNTKVDKKVEPKSC

SEQ ID NO: 53 - protein, 460 aa, Artificial Sequence
  anti-bio antibody full length heavy chain-hole-cys with C-terminal fusion
DKTHTCPPCPAPELLGGPSVFLFPPKPKDTLMISRTPEVTCVVVDVSHEDPEVKFNWYVDGVEVHNAKTKPREEQYNSTYRVVSVLTVLHQDWLNGKEYKCKVSNKALPAPIEKTISKAKGQPREPQVCTLPPSRDELTKNQVSLSCAVKGFYPSDIAVEWESNGQPENNYKTTPPVLDSDGSFFLVSKLTVDKSRWQQGNVFSCSVMHEALHNHYTQKSLSLSPGKGGGGSGGGGSQVQLVQSGAEVKKPGSSVKVSCKSSGFNNKDTFFQWVRQAPGQGLEWMGRIDPANGFTKYAQKFQGRVTITADTSTSTAYMELSSLRSEDTAVYYCARWDTYGAAWFAYWGQGTLVTVSSASTKGPSVFPLAPSSKSTSGGTAALGCLVKDYFPEPVTVSWNSGALTSGVHTFPAVLQSSGLYSLSSVVTVPSSSLGTQTYICNVNHKPSNTKVDKKVEPKSC

SEQ ID NO: 54 - protein, 683 aa, Artificial Sequence
  anti-bio antibody full length heavy chain-hole-cys with N- and C-terminal fusion
QVQLVQSGAEVKKPGSSVKVSCKSSGFNNKDTFFQWVRQAPGQGLEWMGRIDPANGFTKYAQKFQGRVTITADTSTSTAYMELSSLRSEDTAVYYCARWDTYGAAWFAYWGQGTLVTVSSASTKGPSVFPLAPSSKSTSGGTAALGCLVKDYFPEPVTVSWNSGALTSGVHTFPAVLQSSGLYSLSSVVTVPSSSLGTQTYICNVNHKPSNTKVDKKVEPKSCDKTHTCPPCPAPELLGGPSVFLFPPKPKDTLMISRTPEVTCVVVDVSHEDPEVKFNWYVDGVEVHNAKTKPREEQYNSTYRVVSVLTVLHQDWLNGKEYKCKVSNKALPAPIEKTISKAKGQPREPQVCTLPPSRDELTKNQVSLSCAVKGFYPSDIAVEWESNGQPENNYKTTPPVLDSDGSFFLVSKLTVDKSRWQQGNVFSCSVMHEALHNHYTQKSLSLSPGKGGGGSGGGGSQVQLVQSGAEVKKPGSSVKVSCKSSGFNNKDTFFQWVRQAPGQGLEWMGRIDPANGFTKYAQKFQGRVTITADTSTSTAYMELSSLRSEDTAVYYCARWDTYGAAWFAYWGQGTLVTVSSASTKGPSVFPLAPSSKSTSGGTAALGCLVKDYFPEPVTVSWNSGALTSGVHTFPAVLQSSGLYSLSSVVTVPSSSLGTQTYICNVNHKPSNTKVDKKVEPKSC

SEQ ID NO: 55 - protein, 458 aa, Artificial Sequence
  anti-fluos antibody full length heavy chain-hole-cys with C-terminal fusion
DKTHTCPPCPAPELLGGPSVFLFPPKPKDTLMISRTPEVTCVVVDVSHEDPEVKFNWYVDGVEVHNAKTKPREEQYNSTYRVVSVLTVLHQDWLNGKEYKCKVSNKALPAPIEKTISKAKGQPREPQVCTLPPSRDELTKNQVSLSCAVKGFYPSDIAVEWESNGQPENNYKTTPPVLDSDGSFFLVSKLTVDKSRWQQGNVFSCSVMHEALHNHYTQKSLSLSPGKGGGGSGGGGSGVKLDETGGGLVQPGGAMKLSCVTSGFTFGHYWMNWVRQSPEKGLEWVAQFRNKPYNYETYYSDSVKGRFTISRDDSKSSVYLQMNNLRVEDTGIYYCTGASYGMEYLGQGTSVTVSSASTKGPSVFPLAPSSKSTSGGTAALGCLVKDYFPEPVTVSWNSGALTSGVHTFPAVLQSSGLYSLSSVVTVPSSSLGTQTYICNVNHKPSNTKVDKKVEPKSC

SEQ ID NO: 56 - protein, 679 aa, Artificial Sequence
  anti-fluos antibody full length heavy chain-hole-cys with N- and C-terminal fusion
GVKLDETGGGLVQPGGAMKLSCVTSGFTFGHYWMNWVRQSPEKGLEWVAQFRNKPYNYETYYSDSVKGRFTISRDDSKSSVYLQMNNLRVEDTGIYYCTGASYGMEYLGQGTSVTVSSASTKGPSVFPLAPSSKSTSGGTAALGCLVKDYFPEPVTVSWNSGALTSGVHTFPAVLQSSGLYSLSSVVTVPSSSLGTQTYICNVNHKPSNTKVDKKVEPKSCDKTHTCPPCPAPELLGGPSVFLFPPKPKDTLMISRTPEVTCVVVDVSHEDPEVKFNWYVDGVEVHNAKTKPREEQYNSTYRVVSVLTVLHQDWLNGKEYKCKVSNKALPAPIEKTISKAKGQPREPQVCTLPPSRDELTKNQVSLSCAVKGFYPSDIAVEWESNGQPENNYKTTPPVLDSDGSFFLVSKLTVDKSRWQQGNVFSCSVMHEALHNHYTQKSLSLSPGKGGGGSGGGGSGVKLDETGGGLVQPGGAMKLSCVTSGFTFGHYWMNWVRQSPEKGLEWVAQFRNKPYNYETYYSDSVKGRFTISRDDSKSSVYLQMNNLRVEDTGIYYCTGASYGMEYLGQGTSVTVSSASTKGPSVFPLAPSSKSTSGGTAALGCLVKDYFPEPVTVSWNSGALTSGVHTFPAVLQSSGLYSLSSVVTVPSSSLGTQTYICNVNHKPSNTKVDKKVEPKSC

SEQ ID NO: 57 - protein, 450 aa, Artificial Sequence
  anti-bio antibody full length heavy chain-knob without hinge-region cysteine residues
QVQLVQSGAEVKKPGSSVKVSCKSSGFNNKDTFFQWVRQAPGQGLEWMGRIDPANGFTKYAQKFQGRVTITADTSTSTAYMELSSLRSEDTAVYYCARWDTYGAAWFAYWGQGTLVTVSSASTKGPSVFPLAPSSKSTSGGTAALGCLVKDYFPEPVTVSWNSGALTSGVHTFPAVLQSSGLYSLSSVVTVPSSSLGTQTYICNVNHKPSNTKVDKKVEPKSCDKTHTSPPSPAPELLGGPSVFLFPPKPKDTLMISRTPEVTCVVVDVSHEDPEVKFNWYVDGVEVHNAKTKPREEQYNSTYRVVSVLTVLHQDWLNGKEYKCKVSNKALPAPIEKTISKAKGQPREPQVYTLPPSRDELTKNQVSLWCLVKGFYPSDIAVEWESNGQPENNYKTTPPVLDSDGSFFLYSKLTVDKSRWQQGNVFSCSVMHEALHNHYTQKSLSLSPGK

SEQ ID NO: 58 - protein, 450 aa, Artificial Sequence
  anti-bio antibody full length heavy chain-hole without hinge-cysteine residues
QVQLVQSGAEVKKPGSSVKVSCKSSGFNNKDTFFQWVRQAPGQGLEWMGRIDPANGFTKYAQKFQGRVTITADTSTSTAYMELSSLRSEDTAVYYCARWDTYGAAWFAYWGQGTLVTVSSASTKGPSVFPLAPSSKSTSGGTAALGCLVKDYFPEPVTVSWNSGALTSGVHTFPAVLQSSGLYSLSSVVTVPSSSLGTQTYICNVNHKPSNTKVDKKVEPKSCDKTHTSPPSPAPELLGGPSVFLFPPKPKDTLMISRTPEVTCVVVDVSHEDPEVKFNWYVDGVEVHNAKTKPREEQYNSTYRVVSVLTVLHQDWLNGKEYKCKVSNKALPAPIEKTISKAKGQPREPQVYTLPPSRDELTKNQVSLSCAVKGFYPSDIAVEWESNGQPENNYKTTPPVLDSDGSFFLVSKLTVDKSRWQQGNVFSCSVMHEALHNHYTQKSLSLSPGK

SEQ ID NO: 59 - protein, 448 aa, Artificial Sequence
  anti-fluos antibody full length heavy chain-knob without hinge-cysteine residues
GVKLDETGGGLVQPGGAMKLSCVTSGFTFGHYWMNWVRQSPEKGLEWVAQFRNKPYNYETYYSDSVKGRFTISRDDSKSSVYLQMNNLRVEDTGIYYCTGASYGMEYLGQGTSVTVSSASTKGPSVFPLAPSSKSTSGGTAALGCLVKDYFPEPVTVSWNSGALTSGVHTFPAVLQSSGLYSLSSVVTVPSSSLGTQTYICNVNHKPSNTKVDKKVEPKSCDKTHTSPPSPAPELLGGPSVFLFPPKPKDTLMISRTPEVTCVVVDVSHEDPEVKFNWYVDGVEVHNAKTKPREEQYNSTYRVVSVLTVLHQDWLNGKEYKCKVSNKALPAPIEKTISKAKGQPREPQVYTLPPSRDELTKNQVSLWCLVKGFYPSDIAVEWESNGQPENNYKTTPPVLDSDGSFFLYSKLTVDKSRWQQGNVFSCSVMHEALHNHYTQKSLSLSPGK

SEQ ID NO: 60 - protein, 448 aa, Artificial Sequence
  anti-fluos antibody full length heavy chain-hole without hinge-cysteine residues
GVKLDETGGGLVQPGGAMKLSCVTSGFTFGHYWMNWVRQSPEKGLEWVAQFRNKPYNYETYYSDSVKGRFTISRDDSKSSVYLQMNNLRVEDTGIYYCTGASYGMEYLGQGTSVTVSSASTKGPSVFPLAPSSKSTSGGTAALGCLVKDYFPEPVTVSWNSGALTSGVHTFPAVLQSSGLYSLSSVVTVPSSSLGTQTYICNVNHKPSNTKVDKKVEPKSCDKTHTSPPSPAPELLGGPSVFLFPPKPKDTLMISRTPEVTCVVVDVSHEDPEVKFNWYVDGVEVHNAKTKPREEQYNSTYRVVSVLTVLHQDWLNGKEYKCKVSNKALPAPIEKTISKAKGQPREPQVYTLPPSRDELTKNQVSLSCAVKGFYPSDIAVEWESNGQPENNYKTTPPVLDSDGSFFLVSKLTVDKSRWQQGNVFSCSVMHEALHNHYTQKSLSLSPGK

SEQ ID NO: 61 - protein, 240 aa, Artificial Sequence
  MHCFcRP-hole-D356K-His8 without hinge-cysteine residues
DKTHTSPPSPAPELLGGPSVFLFPPKPKDTLMISRTPEVTCVVVDVSHEDPEVKFNWYVDGVEVHNAKTKPREEQYNSTYRVVSVLTVLHQDWLNGKEYKCKVSNKALPAPIEKTISKAKGQPREPQVYTLPPSRKELTKNQVSLSCAVKGFYPSDIAVEWESNGQPENNYKTTPPVLDSDGSFFLVSKLTVDKSRWQQGNVFSCSVMHEALHNHYTQKSLSLSPGKGGGGSHHHHHHHH

SEQ ID NO: 62 - protein, 240 aa, Artificial Sequence
  MHCFcRP-hole-E357K-His8 without hinge-cysteine residues
DKTHTSPPSPAPELLGGPSVFLFPPKPKDTLMISRTPEVTCVVVDVSHEDPEVKFNWYVDGVEVHNAKTKPREEQYNSTYRVVSVLTVLHQDWLNGKEYKCKVSNKALPAPIEKTISKAKGQPREPQVYTLPPSRDKLTKNQVSLSCAVKGFYPSDIAVEWESNGQPENNYKTTPPVLDSDGSFFLVSKLTVDKSRWQQGNVFSCSVMHEALHNHYTQKSLSLSPGKGGGGSHHHHHHHH

SEQ ID NO: 63 - protein, 240 aa, Artificial Sequence
  MHCFcRP-knob-K370E-His8 without hinge-cysteine residues
DKTHTSPPSPAPELLGGPSVFLFPPKPKDTLMISRTPEVTCVVVDVSHEDPEVKFNWYVDGVEVHNAKTKPREEQYNSTYRVVSVLTVLHQDWLNGKEYKCKVSNKALPAPIEKTISKAKGQPREPQVYTLPPSRDELTKNQVSLWCLVEGFYPSDIAVEWESNGQPENNYKTTPPVLDSDGSFFLYSKLTVDKSRWQQGNVFSCSVMHEALHNHYTQKSLSLSPGKGGGGSHHHHHHHH

SEQ ID NO: 64 - protein, 240 aa, Artificial Sequence
  MHCFcRP-knob-K439E-His8 without hinge-cysteine residues
DKTHTSPPSPAPELLGGPSVFLFPPKPKDTLMISRTPEVTCVVVDVSHEDPEVKFNWYVDGVEVHNAKTKPREEQYNSTYRVVSVLTVLHQDWLNGKEYKCKVSNKALPAPIEKTISKAKGQPREPQVYTLPPSRDELTKNQVSLWCLVKGFYPSDIAVEWESNGQPENNYKTTPPVLDSDGSFFLYSKLTVDKSRWQQGNVFSCSVMHEALHNHYTQESLSLSPGKGGGGSHHHHHHHH

SEQ ID NO: 65 - protein, 9 aa, Homo sapiens
DKTHTCPPC

SEQ ID NO: 66 - protein, 9 aa, Artificial Sequence
  cys-free hinge region
DKTHTSPPS

SEQ ID NO: 67 - protein, 6 aa, Artificial Sequence
  hexa-histidine tag
HHHHHH

SEQ ID NO: 68 - protein, 8 aa, Artificial Sequence
  octa-histidine tag
HHHHHHHH

SEQ ID NO: 69 - protein, 4 aa, Artificial Sequence
  peptidic linker
GGGS

SEQ ID NO: 70 - protein, 5 aa, Artificial Sequence
  peptidic linker
GGGGS

SEQ ID NO: 71 - protein, 4 aa, Artificial Sequence
  peptidic linker
QQQS

SEQ ID NO: 72 - protein, 5 aa, Artificial Sequence
  peptidic linker
QQQQS

SEQ ID NO: 73 - protein, 4 aa, Artificial Sequence
  peptidic linker
SSSG

SEQ ID NO: 74 - protein, 5 aa, Artificial Sequence
  peptidic linker
SSSSG

SEQ ID NO: 75 - protein, 8 aa, Artificial Sequence
  peptidic linker
GGGSGGGS

SEQ ID NO: 76 - protein, 12 aa, Artificial Sequence
  peptidic linker
GGGSGGGSGGGS

SEQ ID NO: 77 - protein, 16 aa, Artificial Sequence
  peptidic linker
GGGSGGGSGGGSGGGS

SEQ ID NO: 78 - protein, 20 aa, Artificial Sequence
  peptidic linker
GGGSGGGSGGGSGGGSGGGS

SEQ ID NO: 79 - protein, 10 aa, Artificial Sequence
  peptidic linker
GGGGSGGGGS

SEQ ID NO: 80 - protein, 15 aa, Artificial Sequence
  peptidic linker
GGGGSGGGGSGGGGS

SEQ ID NO: 81 - protein, 20 aa, Artificial Sequence
  peptidic linker
GGGGSGGGGSGGGGSGGGGS

SEQ ID NO: 82 - protein, 17 aa, Artificial Sequence
  peptidic linker
GSSSSSSSSSSSSSSSG

SEQ ID NO: 83 - protein, 227 aa, Artificial Sequence
  affibody-MHCFcRP
DIQMTQSPSSLSASVGDRVTITCRASGNIHNYLSWYQQKPGKVPKLLIYSAKTLADGVPSRFSGSGSGTDFTLTISSLQPEDVATYYCQHFWSSIYTFGQGTKLEIKGQPREPQVYTLPPSRDKLTKNQVSLSCAVKGFYPSDIAVEWESNGQPENNYKTTPPVLDSDGSFFLVSKLTVDKSRWQQGNVFSCSVMHEALHNHYTQKSLSLSPGKGGGGSHHHHHHHH

SEQ ID NO: 84 - protein, 306 aa, Artificial Sequence
  affibody-VH
VDNKFNKEMRNAYWEIALLPNLNNQQKRAFIRSLYDDPSQSANLLAEAKKLNDAQAPKGTGGGGSGGGGSGGGGSGGGGSEVQLVQSGAEVKKPGASVKVSCKASGYTFTNYYIHWVRQAPGQGLEWIGWIYPGDGNTKYNEKFKGRATLTADTSTSTAYLELSSLRSEDTAVYYCARDSYSNYYFDYWGQGTLVTVSSGQPREPQVYTLPPSRDELTKNQVSLWCLVKGFYPSDIAVEWESNGQPENNYKTTPPVLDSDGSFFLYSKLTVDKSRWQQGNVFSCSVMHEALHNHYTQKSLSLSPGK

SEQ ID NO: 85 - protein, 7 aa, Artificial Sequence
  hinge region
  MISC_FEATURE (5)..(5): X=S or P
HTSPXSP

SEQ ID NO: 86 - protein, 6 aa, Artificial Sequence
  hinge region#
HTPAPE

SEQ ID NO: 87 - protein, 4 aa, Artificial Sequence
  C-tag
EPEA

SEQ ID NO: 88 - protein, 9 aa, Artificial Sequence
  C-tag with linker
GGGGSEPEA

SEQ ID NO: 89 - protein, 4 aa, Homo sapiens
  MISC_FEATURE (3)..(3): X = S or P
CPXC

SEQ ID NO: 90 - protein, 10 aa, Homo sapiens
HTCPPCPAPE

SEQ ID NO: 91 - protein, 5 aa, Homo sapiens
DKTHT